European Patent Application EP 4 786 599 A1, published August 5, 2026. Title: 具有细胞内信号传导结构域及自然杀伤蛋白30跨膜结构域的核酸分子及包含其的嵌合抗原受体. Applicant: 沛尔生技医药股份有限公司. The sequence listing filed with the application follows.

SEQUENCE LISTING (99 sequences)

SEQ ID NO: 1 - protein, 242 aa, synthetic construct
  SITE 1..242: note = anti BCMA VHH1-GGGGS -VHH2
QVKLEESGGGLVQAGRSLRLSCAASEHTFSSHVMGWFRQAPGKERESVAVIGWRDISTSYADSVKGRFTISRDNAKKTLYLQMNSLKPEDTAVYYCAARRIDAADFDSWGQGTQVTVSSGGGGSEVQLVESGGGLVQAGGSLRLSCAASGRTFTMGWFRQAPGKEREFVAAISLSPTLAYYAESVKGRFTISRDNAKNTVVLQMNSLKPEDTALYYCAADRKSVMSIRPDYWGQGTQVTVSS

SEQ ID NO: 2 - protein, 119 aa, synthetic construct
  SITE 1..119: note = anti BCMA VHH1
QVKLEESGGGLVQAGRSLRLSCAASEHTFSSHVMGWFRQAPGKERESVAVIGWRDISTSYADSVKGRFTISRDNAKKTLYLQMNSLKPEDTAVYYCAARRIDAADFDSWGQGTQVTVSS

SEQ ID NO: 3 - protein, 118 aa, synthetic construct
  SITE 1..118: note = anti BCMA VHH2
EVQLVESGGGLVQAGGSLRLSCAASGRTFTMGWFRQAPGKEREFVAAISLSPTLAYYAESVKGRFTISRDNAKNTVVLQMNSLKPEDTALYYCAADRKSVMSIRPDYWGQGTQVTVSS

SEQ ID NO: 4 - protein, 9 aa, synthetic construct
  SITE 1..9: note = anti BCMA VHH1 CDRH1
HTFSSHVMG

SEQ ID NO: 5 - protein, 11 aa, synthetic construct
  SITE 1..11: note = anti BCMA VHH1 CDRH2
GWRDISTSYAD

SEQ ID NO: 6 - protein, 12 aa, synthetic construct
  SITE 1..12: note = anti BCMA VHH1 CDRH3
AARRIDAADFDS

SEQ ID NO: 7 - protein, 6 aa, synthetic construct
  SITE 1..6: note = anti BCMA VHH2 CDRH1
RTFTMG

SEQ ID NO: 8 - protein, 11 aa, synthetic construct
  SITE 1..11: note = anti BCMA VHH2 CDRH2
SLSPTLAYYAE

SEQ ID NO: 9 - protein, 14 aa, synthetic construct
  SITE 1..14: note = anti BCMA VHH2 CDRH3
AADRKSVMSIRPDY

SEQ ID NO: 10 - protein, 10 aa, synthetic construct
  SITE 1..10: note = anti CD19 antibody(FMC63) CDRH1
GVSLPDYGVS

SEQ ID NO: 11 - protein, 16 aa, synthetic construct
  SITE 1..16: note = anti CD19 antibody(FMC63) CDRH2
VIWGSETTYYNSALKS

SEQ ID NO: 12 - protein, 12 aa, synthetic construct
  SITE 1..12: note = anti CD19 antibody(FMC63) CDRH3
HYYYGGSYAMDY

SEQ ID NO: 13 - protein, 11 aa, synthetic construct
  SITE 1..11: note = anti CD19 antibody(FMC63) CDRL1
RASQDISKYLN

SEQ ID NO: 14 - protein, 7 aa, synthetic construct
  SITE 1..7: note = anti CD19 antibody(FMC63) CDRL2
SRLHSGV

SEQ ID NO: 15 - protein, 9 aa, synthetic construct
  SITE 1..9: note = anti CD19 antibody(FMC63) CDRL3
QQGNTLPYT

SEQ ID NO: 16 - protein, 242 aa, synthetic construct
  SITE 1..242: note = FMC63 scfv
DIQMTQTTSSLSASLGDRVTISCRASQDISKYLNWYQQKPDGTVKLLIYHTSRLHSGVPSRFSGSGSGTDYSLTISNLEQEDIATYFCQQGNTLPYTFGGGTKLEITGGGGSGGGGSGGGGSEVKLQESGPGLVAPSQSLSVTCTVSGVSLPDYGVSWIRQPPRKGLEWLGVIWGSETTYYNSALKSRLTIIKDNSKSQVFLKMNSLQTDDTAIYYCAKHYYYGGSYAMDYWGQGTSVTVSS

SEQ ID NO: 17 - protein, 5 aa, synthetic construct
  SITE 1..5: note = anti mesothelin antibody(SS1) CDRH1
GYTMN

SEQ ID NO: 18 - protein, 15 aa, synthetic construct
  SITE 1..15: note = anti mesothelin antibody(SS1) CDRH2
LITPYNGASSYNQKF

SEQ ID NO: 19 - protein, 10 aa, synthetic construct
  SITE 1..10: note = anti mesothelin antibody(SS1) CDRH3
GGYDGRGFDY

SEQ ID NO: 20 - protein, 10 aa, synthetic construct
  SITE 1..10: note = anti mesothelin antibody(SS1) CDRL1
SASSSVSYMH

SEQ ID NO: 21 - protein, 7 aa, synthetic construct
  SITE 1..7: note = anti mesothelin antibody(SS1) CDRL2
DTSKLAS

SEQ ID NO: 22 - protein, 9 aa, synthetic construct
  SITE 1..9: note = anti mesothelin antibody(SS1) CDRL3
QQWSKHPLT

SEQ ID NO: 23 - protein, 240 aa, synthetic construct
  SITE 1..240: note = SS1 scfv
QVQLQQSGPELEKPGASVKLSCKASGYSFTGYTMNWVKQSHGKSLEWIGLITPYNGASSYNQKFRGKATLTVDKSSSTAYMDLLSLTSEDSAVYFCARGGYDGRGFDYWGQGTTVTVSSGVGGSGGGGSGGGGSDIELTQSPAIMSASPGEKVTMTCSASSSVSYMHWYQQKSGTSPKRWIYDTSKLASGVPGRFSGSGSGNSYSLTISSVEAEDDATYYCQQWSKHPLTFGAGTKLEIK

SEQ ID NO: 24 - protein, 10 aa, synthetic construct
  SITE 1..10: note = anti BCMA antibody(J6M0) CDRH1
GGTFSNYWMH

SEQ ID NO: 25 - protein, 17 aa, synthetic construct
  SITE 1..17: note = anti BCMA antibody(J6M0) CDRH2
ATYRGHSDTYYNQKFKG

SEQ ID NO: 26 - protein, 12 aa, synthetic construct
  SITE 1..12: note = anti BCMA antibody(J6M0) CDRH3
GAIYDGYDVLDN

SEQ ID NO: 27 - protein, 11 aa, synthetic construct
  SITE 1..11: note = anti BCMA antibody(J6M0) CDRL1
SASQDISNYLN

SEQ ID NO: 28 - protein, 7 aa, synthetic construct
  SITE 1..7: note = anti BCMA antibody(J6M0) CDRL2
YTSNLHS

SEQ ID NO: 29 - protein, 9 aa, synthetic construct
  SITE 1..9: note = anti BCMA antibody(J6M0) CDRL3
QQYRKLPWT

SEQ ID NO: 30 - protein, 244 aa, synthetic construct
  SITE 1..244: note = J6M0 scfv
QVQLVQSGAEVKKPGSSVKVSCKASGGTFSNYWMHWVRQAPGQGLEWMGATYRGHSDTYYNQKFKGRVTITADKSTSTAYMELSSLRSEDTAVYYCARGAIYDGYDVLDNWGQGTLVTVSSGGGGSGGGGSGGGGSDIQMTQSPSSLSASVGDRVTITCSASQDISNYLNWYQQKPGKAPKLLIYYTSNLHSGVPSRFSGSGSGTDFTLTISSLQPEDFATYYCQQYRKLPWTFGQGTKLEIKR

SEQ ID NO: 31 - protein, 10 aa, synthetic construct
  SITE 1..10: note = anti BCMA antibody(BB2121) CDRH1
GYTFTDYSIN

SEQ ID NO: 32 - protein, 17 aa, synthetic construct
  SITE 1..17: note = anti BCMA antibody(BB2121) CDRH2
WINTETREPAYAYDFRG

SEQ ID NO: 33 - protein, 8 aa, synthetic construct
  SITE 1..8: note = anti BCMA antibody(BB2121) CDRH3
DYSYAMDY

SEQ ID NO: 34 - protein, 15 aa, synthetic construct
  SITE 1..15: note = anti BCMA antibody(BB2121) CDRL1
RASESVTILGSHLIH

SEQ ID NO: 35 - protein, 7 aa, synthetic construct
  SITE 1..7: note = anti BCMA antibody(BB2121) CDRL2
LASNVQT

SEQ ID NO: 36 - protein, 8 aa, synthetic construct
  SITE 1..8: note = anti BCMA antibody(BB2121) CDRL3
QSRTIPRT

SEQ ID NO: 37 - protein, 246 aa, synthetic construct
  SITE 1..246: note = BB2121 scfv
DIVLTQSPPSLAMSLGKRATISCRASESVTILGSHLIHWYQQKPGQPPTLLIQLASNVQTGVPARFSGSGSRTDFTLTIDPVEEDDVAVYYCLQSRTIPRTFGGGTKLEIKGSTSGSGKPGSGEGSTKGQIQLVQSGPELKKPGETVKISCKASGYTFTDYSINWVKRAPGKGLKWMGWINTETREPAYAYDFRGRFAFSLETSASTAYLQINNLKYEDTATYFCALDYSYAMDYWGQGTSVTVSS

SEQ ID NO: 38 - protein, 8 aa, synthetic construct
  SITE 1..8: note = anti CD22 antibody(m971) CDRH1
SSNSAAWN

SEQ ID NO: 39 - protein, 18 aa, synthetic construct
  SITE 1..18: note = anti CD22 antibody(m971) CDRH2
RTYYRSKWYNDYAVSVKS

SEQ ID NO: 40 - protein, 12 aa, synthetic construct
  SITE 1..12: note = anti CD22 antibody(m971) CDRH3
EVTGDLEDAFDI

SEQ ID NO: 41 - protein, 10 aa, synthetic construct
  SITE 1..10: note = anti CD22 antibody(m971) CDRL1
RASQTIWSYL

SEQ ID NO: 42 - protein, 7 aa, synthetic construct
  SITE 1..7: note = anti CD22 antibody(m971) CDRL2
AASSLQS

SEQ ID NO: 43 - protein, 9 aa, synthetic construct
  SITE 1..9: note = anti CD22 antibody(m971) CDRL3
QQSYSIPQT

SEQ ID NO: 44 - protein, 246 aa, synthetic construct
  SITE 1..246: note = m971 scfv
QVQLQQSGPGLVKPSQTLSLTCAISGDSVSSNSAAWNWIRQSPSRGLEWLGRTYYRSKWYNDYAVSVKSRITINPDTSKNQFSLQLNSVTPEDTAVYYCAREVTGDLEDAFDIWGQGTMVTVSSGGGGSGGGGSGGGGSDIQMTQSPSSLSASVGDRVTITCRASQTIWSYLNWYQQRPGKAPNLLIYAASSLQSGVPSRFSGRGSGTDFTLTISSLQAEDFATYYCQQSYSIPQTFGQGTKLEIK

SEQ ID NO: 45 - protein, 10 aa, synthetic construct
  SITE 1..10: note = anti CD22 antibody(LL2) CDRH1
GYTFTSYWLH

SEQ ID NO: 46 - protein, 17 aa, synthetic construct
  SITE 1..17: note = anti CD22 antibody(LL2) CDRH2
YINPRNDYTEYNQNFKD

SEQ ID NO: 47 - protein, 7 aa, synthetic construct
  SITE 1..7: note = anti CD22 antibody(LL2) CDRH3
RDITIFY

SEQ ID NO: 48 - protein, 16 aa, synthetic construct
  SITE 1..16: note = anti CD22 antibody(LL2) CDRL1
KSSQSVLYSANHKNYL

SEQ ID NO: 49 - protein, 7 aa, synthetic construct
  SITE 1..7: note = anti CD22 antibody(LL2) CDRL2
WASTRES

SEQ ID NO: 50 - protein, 8 aa, synthetic construct
  SITE 1..8: note = anti CD22 antibody(LL2) CDRL3
HQTLSSWT

SEQ ID NO: 51 - protein, 244 aa, synthetic construct
  SITE 1..244: note = LL2 scfv
QVQLVQSGAEVKKPGSSVKVSCKASGYTFTSYWLHWVRQAPGQGLEWIGYINPRNDYTEYNQNFKDKATITADESTNTAYMELSSLRSEDTAFYFCARRDITTFYWGQGTTVTVSSGGGGSGGGGSGGGGSDIQLTQSPSSLSASVGDRVTMSCKSSQSVLYSANHKNYLAWYQQKPGKAPKLLIYWASTRESGVPSRFSGSGSGTDFTFTISSLQPEDIATYYCHQYLSSWTFGGGTKLEIKR

SEQ ID NO: 52 - protein, 10 aa, synthetic construct
  SITE 1..10: note = anti CD22 antibody(G5/44) CDRH1
GYRFTNYWIH

SEQ ID NO: 53 - protein, 17 aa, synthetic construct
  SITE 1..17: note = anti CD22 antibody(G5/44) CDRH2
GINPGNNYATYRRKFQG

SEQ ID NO: 54 - protein, 12 aa, synthetic construct
  SITE 1..12: note = anti CD22 antibody(G5/44) CDRH3
EGYGNYGAWFAY

SEQ ID NO: 55 - protein, 15 aa, synthetic construct
  SITE 1..15: note = anti CD22 antibody(G5/44) CDRL1
RSSQSLANSYGNTFL

SEQ ID NO: 56 - protein, 7 aa, synthetic construct
  SITE 1..7: note = anti CD22 antibody(G5/44) CDRL2
GISNRFS

SEQ ID NO: 57 - protein, 9 aa, synthetic construct
  SITE 1..9: note = anti CD22 antibody(G5/44) CDRL3
LQGTHQPYT

SEQ ID NO: 58 - protein, 249 aa, synthetic construct
  SITE 1..249: note = G5/44 scfv
EVQLVQSGAEVKKPGASVKVSCKASGYRFTNYWIHWVRQAPGQGLEWIGGINPGNNYATYRRKFQGRVTMTADTSTSTVYMELSSLRSEDTAVYYCTREGYGNYGAWFAYWGQGTLVTVSSGGGGSGGGGSGGGGSDVQVTQSPSSLSASVGDRVTITCRSSQSLANSYGNTFLSWYLHKPGKAPQLLIYGISNRFSGVPDRFSGSGSGTDFTLTISSLQPEDFATYYCLQGTHQPYTFGQGTKVEIKR

SEQ ID NO: 59 - protein, 10 aa, synthetic construct
  SITE 1..10: note = anti CD22 antibody(RFB4) CDRH1
GFTFSIYDMS

SEQ ID NO: 60 - protein, 17 aa, synthetic construct
  SITE 1..17: note = anti CD22 antibody(RFB4) CDRH2
YISSGGGTTYYPDTVKG

SEQ ID NO: 61 - protein, 14 aa, synthetic construct
  SITE 1..14: note = anti CD22 antibody(RFB4) CDRH3
HSGYGSSYGVLFAY

SEQ ID NO: 62 - protein, 10 aa, synthetic construct
  SITE 1..10: note = anti CD22 antibody(RFB4) CDRL1
RASQTISNYL

SEQ ID NO: 63 - protein, 7 aa, synthetic construct
  SITE 1..7: note = anti CD22 antibody(RFB4) CDRL2
YTSILHS

SEQ ID NO: 64 - protein, 9 aa, synthetic construct
  SITE 1..9: note = anti CD22 antibody(RFB4) CDRL3
QQGNTLPWT

SEQ ID NO: 65 - protein, 244 aa, synthetic construct
  SITE 1..244: note = RFB4 scfv
QLVQSGAEVKKPGSSVKVSCKASGFTFSIYDMSWVRQAPGQGLEWVAYISSGGGTTYYPDTVKGRFTITADESTNTAYMELSSLRSEDTAFYFCARHSGYGSSYGVLFAYWGQGTLVTVSSGGGGSGGGGSGGGGSDIQLTQSPSSLSASVGDRVTISCRASQDISNYLNWYQQKPGKAPKLLIYYTSILHSGVPSRFSGSGSGTDYTFTISSLQPEDIATYYCQQGNTLPWTFGGGTKVQIKR

SEQ ID NO: 66 - DNA, 45 bp, synthetic construct
  source 1..45: mol_type = other DNA
  misc_feature 1..45: note = (G4S)3 hinge
ggcggcggaggctctggcggcggcggcagcggcggcggaggctcc

SEQ ID NO: 67 - DNA, 207 bp, synthetic construct
  source 1..207: mol_type = other DNA
  misc_feature 1..207: note = CD8 hinge
accactaccccagcaccgaggccacccaccccggctcctaccatcgcctcccagcctctgtccctgcgtccggaggcatgtagacccgcagctggtggggccgtgcatacccggggtcttgacttcgcctgcgatatctacatttgggcccctctggctggtacttgcggggtcctgctgctttcactcgtgatcactctttactgt

SEQ ID NO: 68 - DNA, 117 bp, synthetic construct
  source 1..117: mol_type = other DNA
  misc_feature 1..117: note = CD28 hinge
attgaagttatgtatcctcctccttacctagacaatgagaagagcaatggaaccattatccatgtgaaagggaaacacctttgtccaagtcccctatttcccggaccttctaagccc

SEQ ID NO: 69 - DNA, 36 bp, synthetic construct
  source 1..36: mol_type = other DNA
  misc_feature 1..36: note = IgG4 hinge
gagtccaaatatggtcccccatgcccatcatgccca

SEQ ID NO: 70 - DNA, 30 bp, synthetic construct
  source 1..30: mol_type = other DNA
  misc_feature 1..30: note = EAAAKGGGGS hinge
gaagcggcggcgaaaggaggaggaggaagc

SEQ ID NO: 71 - DNA, 45 bp, synthetic construct
  source 1..45: mol_type = other DNA
  misc_feature 1..45: note = (EAAAK)3 hinge
gaagcagccgctaaagaggcagctgctaaggaagccgcagctaaa

SEQ ID NO: 72 - DNA, 54 bp, synthetic construct
  source 1..54: mol_type = other DNA
  misc_feature 1..54: note = GST hinge
ggaagcacgtccggctcagggaagccgggctccggcgagggaagcacgaagggg

SEQ ID NO: 73 - DNA, 60 bp, synthetic construct
  source 1..60: mol_type = other DNA
  misc_feature 1..60: note = EAAAK-GS hinge
gaagcagccgctaaaggcggaggcggttctggaggcggtggctccgcggccgcagctaag

SEQ ID NO: 74 - DNA, 192 bp, synthetic construct
  source 1..192: mol_type = other DNA
  misc_feature 1..192: note = IgD hinge
aggtggcccgaaagtcccaaggcccaggcatctagtgttcctactgcacagccccaggcagaaggcagcctagccaaagctactactgcacctgccactacgcgcaatactggccgtggcggggaggagaagaaaaaggagaaagagaaagaagaacaggaagagagggagaccaagacccctgaatgtcca

SEQ ID NO: 75 - DNA, 357 bp, synthetic construct
  source 1..357: mol_type = other DNA
  misc_feature 1..357: note = IgG4-CH3 hinge
gagtccaaatatggtcccccatgcccatcatgcccagggcagccccgagagccacaggtgtacaccctgcccccatcccaggaggagatgaccaagaaccaggtcagcctgacctgcctggtcaaaggcttctaccccagcgacatcgccgtggagtgggagagcaatgggcagccggagaacaactacaagaccacgcctcccgtgctggactccgacggctccttcttcctctacagcaggctaaccgtggacaagagcaggtggcaggaggggaatgtcttctcatgctccgtgatgcatgaggctctgcacaaccactacacacagaagagcctctccctgtctctgggtaaa

SEQ ID NO: 76 - DNA, 36 bp, synthetic construct
  source 1..36: mol_type = other DNA
  misc_feature 1..36: note = (AP)6 hinge
gcacctgcccctgcaccagctccagctcccgcccca

SEQ ID NO: 77 - DNA, 258 bp, synthetic construct
  source 1..258: mol_type = other DNA
  misc_feature 1..258: note = DNA sequence of Fc epsilon R1 gamma
atgattccagcagtggtcttgctcttactccttttggttgaacaagcagcggccctgggagagcctcagctctgctatatcctggatgccatcctgtttctgtatggaattgtcctcaccctcctctactgtcgactgaagatccaagtgcgaaaggcagctataaccagctatgagaaatcagatggtgtttacacgggcctgagcaccaggaaccaggagacttacgagactctgaagcatgagaaaccaccacag

SEQ ID NO: 78 - DNA, 156 bp, synthetic construct
  source 1..156: mol_type = other DNA
  misc_feature 1..156: note = DNA sequence of DAP12 intracellular signaling domain
tacttcctgggccggctggtccctcgggggcgaggggctgcggaggcagcgacccggaaacagcgtatcactgagaccgagtcgccttatcaggagctccagggtcagaggtcggatgtctacagcgacctcaacacacagaggccgtattacaaa

SEQ ID NO: 79 - DNA, 612 bp, synthetic construct
  source 1..612: mol_type = other DNA
  misc_feature 1..612: note = NKp30 (DNA sequence)
atggcctggatgctgctgctgatcctgatcatggtgcaccctggctcttgcgcactgtgggtgagccagccaccagagatccgcacactggagggcagctccgccttcctgccatgttcctttaacgcatctcagggccggctggcaatcggctccgtgacctggtttagagacgaggtggtgcccggcaaggaggtgaggaatggcacacccgagttcaggggccgcctggcacctctggcctctagccggtttctgcacgatcaccaggccgagctgcacatccgggacgtgagaggccacgatgcctctatctacgtgtgccgggtggaggtgctgggcctgggagtgggcaccggcaacggcacacggctggtggtggagaaggagcaccctcagctgggagcaggcaccgtgctgctgctgagggccggcttctatgccgtgagctttctgtccgtggccgtgggctccaccgtgtactatcagggcaagtgcctgacatggaaaggcccccggagacagctgccagccgtggtgccagcaccactgcctccaccctgtggctcctctgcccacctgctgcctccagtgcccggcggctgagaattc

SEQ ID NO: 80 - DNA, 63 bp, synthetic construct
  source 1..63: mol_type = other DNA
  misc_feature 1..63: note = T2A (DNA sequence)
ggctctggagagggaagaggcagcctgctgacctgcggcgacgtggaggagaatcctggccca

SEQ ID NO: 81 - DNA, 1101 bp, synthetic construct
  source 1..1101: mol_type = other DNA
  misc_feature 1..1101: note = the nucleic acid molecule of example 1-1
ttcgaagccaccatgatcccagccgtggtgctgctgctgctgctgctggtggagcaggccgccgccctgggagagccccagctgtgctacatcctggacgccatcctgttcctgtacggcatcgtgctgaccctgctgtattgtaggctgaagatccaggtgcgcaaggccgccatcacatcttacgagaagagcgatggcgtgtataccggcctgagcacaagaaaccaggagacatacgagacactgaagcacgagaagccacctcagtacttcctgggccggctggtgccaaggggaagaggagcagcagaggcagccaccaggaagcagcgcatcaccgagacagagtctccataccaggagctgcagggacagcggagcgacgtgtattccgatctgaacacacagaggccttactataagggcagcggagagggaaggggctccctgctgacctgcggcgacgtggaggagaatcccggccctatggcctggatgctgctgctgatcctgatcatggtgcaccctggctcttgcgcactgtgggtgagccagccaccagagatccgcacactggagggcagctccgccttcctgccatgttcctttaacgcatctcagggccggctggcaatcggctccgtgacctggtttagagacgaggtggtgcccggcaaggaggtgaggaatggcacacccgagttcaggggccgcctggcacctctggcctctagccggtttctgcacgatcaccaggccgagctgcacatccgggacgtgagaggccacgatgcctctatctacgtgtgccgggtggaggtgctgggcctgggagtgggcaccggcaacggcacacggctggtggtggagaaggagcaccctcagctgggagcaggcaccgtgctgctgctgagggccggcttctatgccgtgagctttctgtccgtggccgtgggctccaccgtgtactatcagggcaagtgcctgacatggaaaggcccccggagacagctgccagccgtggtgccagcaccactgcctccaccctgtggctcctctgcccacctgctgcctccagtgcccggcggctgagaattc

SEQ ID NO: 82 - DNA, 126 bp, synthetic construct
  source 1..126: mol_type = other DNA
  misc_feature 1..126: note = 41BB intracellular signaling domain (DNA sequence)
aagcgcggtcggaagaagctgctgtacatctttaagcaacccttcatgaggcctgtgcagactactcaagaggaggacggctgttcatgccggttcccagaggaggaggaaggcggctgcgaactg

SEQ ID NO: 83 - DNA, 1071 bp, synthetic construct
  source 1..1071: mol_type = other DNA
  misc_feature 1..1071: note = the nucleic acid molecule of example 1-2
ttcgaagccaccatgatcccagccgtggtgctgctgctgctgctgctggtggagcaggccgccgccctgggagagccccagctgtgctacatcctggacgccatcctgttcctgtacggcatcgtgctgaccctgctgtattgtaggctgaagatccaggtgcgcaaggccgccatcacatcttacgagaagagcgatggcgtgtataccggcctgagcacaagaaaccaggagacatacgagacactgaagcacgagaagccacctcagaagcgcggtcggaagaagctgctgtacatctttaagcaacccttcatgaggcctgtgcagactactcaagaggaggacggctgttcatgccggttcccagaggaggaggaaggcggctgcgaactgggctctggagagggaagaggcagcctgctgacctgcggcgacgtggaggagaatcctggcccaatggcctggatgctgctgctgatcctgatcatggtgcaccctggctcttgcgcactgtgggtgagccagccaccagagatccgcacactggagggcagctccgccttcctgccatgttcctttaacgcatctcagggccggctggcaatcggctccgtgacctggtttagagacgaggtggtgcccggcaaggaggtgaggaatggcacacccgagttcaggggccgcctggcacctctggcctctagccggtttctgcacgatcaccaggccgagctgcacatccgggacgtgagaggccacgatgcctctatctacgtgtgccgggtggaggtgctgggcctgggagtgggcaccggcaacggcacacggctggtggtggagaaggagcaccctcagctgggagcaggcaccgtgctgctgctgagggccggcttctatgccgtgagctttctgtccgtggccgtgggctccaccgtgtactatcagggcaagtgcctgacatggaaaggcccccggagacagctgccagccgtggtgccagcaccactgcctccaccctgtggctcctctgcccacctgctgcctccagtgcccggcggctgagaattc

SEQ ID NO: 84 - DNA, 945 bp, synthetic construct
  source 1..945: mol_type = other DNA
  misc_feature 1..945: note = the nucleic acid molecule of comparative example 1
ttcgaagccaccatgatcccagccgtggtgctgctgctgctgctgctggtggagcaggccgccgccctgggagagccccagctgtgctacatcctggacgccatcctgttcctgtacggcatcgtgctgaccctgctgtattgtaggctgaagatccaggtgcgcaaggccgccatcacatcttacgagaagagcgatggcgtgtataccggcctgagcacaagaaaccaggagacatacgagacactgaagcacgagaagccacctcagggctctggagagggaagaggcagcctgctgacctgcggcgacgtggaggagaatcctggcccaatggcctggatgctgctgctgatcctgatcatggtgcaccctggctcttgcgcactgtgggtgagccagccaccagagatccgcacactggagggcagctccgccttcctgccatgttcctttaacgcatctcagggccggctggcaatcggctccgtgacctggtttagagacgaggtggtgcccggcaaggaggtgaggaatggcacacccgagttcaggggccgcctggcacctctggcctctagccggtttctgcacgatcaccaggccgagctgcacatccgggacgtgagaggccacgatgcctctatctacgtgtgccgggtggaggtgctgggcctgggagtgggcaccggcaacggcacacggctggtggtggagaaggagcaccctcagctgggagcaggcaccgtgctgctgctgagggccggcttctatgccgtgagctttctgtccgtggccgtgggctccaccgtgtactatcagggcaagtgcctgacatggaaaggcccccggagacagctgccagccgtggtgccagcaccactgcctccaccctgtggctcctctgcccacctgctgcctccagtgcccggcggctgagaattc

SEQ ID NO: 85 - DNA, 720 bp, synthetic construct
  source 1..720: mol_type = other DNA
  misc_feature 1..720: note = SS1 scfv
caggtgcagctccagcagtccggcccagagctggagaagcctggcgcctctgtgaagctgagctgtaaggccagcggctactccttcaccggctatacaatgaactgggtgaagcagtcccacggcaagtctctggagtggatcggcctgatcaccccctacaacggcgccagctcctataatcagaagtttcgcggcaaggccaccctgacagtggataagtctagctccaccgcctacatggacctgctgtctctgacaagcgaggattccgccgtgtacttctgcgccagaggcggctatgacggcagaggctttgattactggggccagggcaccacagtgaccgtgtctagcggcgtgggcggctctggaggaggaggcagcggcggaggaggctccgacatcgagctgacacagtccccagcaatcatgtctgccagccccggcgagaaggtgaccatgacatgttccgcctcctctagcgtgtcttacatgcactggtatcagcagaagtctggcaccagccctaagaggtggatctatgatacaagcaagctggcatccggcgtgccaggccgcttctccggctctggcagcggcaattcctactctctgaccatctcctctgtggaggccgaggacgatgccacatactattgccagcagtggagcaagcacccactgacctttggcgccggcacaaagctggagatcaag

SEQ ID NO: 86 - DNA, 225 bp, synthetic construct
  source 1..225: mol_type = other DNA
  misc_feature 1..225: note = NKp30 without Ig-like domain (DNA sequence)
gtggagaaggagcaccctcagctgggagcaggcaccgtgctgctgctgagggccggcttctatgccgtgagctttctgtccgtggccgtgggctccaccgtgtactatcagggcaagtgcctgacatggaaaggcccccggagacagctgccagccgtggtgccagcaccactgcctccaccctgtggctcctctgcccacctgctgcctccagtgcccggcggc

SEQ ID NO: 87 - DNA, 1566 bp, synthetic construct
  source 1..1566: mol_type = other DNA
  misc_feature 1..1566: note = the nucleic acid molecule of example 2
atgattccagcagtggtcttgctcttactccttttggttgaacaagcagcggccctgggagagcctcagctctgctatatcctggatgccatcctgtttctgtatggaattgtcctcaccctcctctactgtcgactgaagatccaagtgcgaaaggcagctataaccagctatgagaaatcagatggtgtttacacgggcctgagcaccaggaaccaggagacttacgagactctgaagcatgagaaaccaccacagggctctggagagggaagaggcagcctgctgacctgcggcgacgtggaggagaatcctggcccaatcgatgccaccatcgatgccaccatggccttaccagtgaccgccttgctcctgccgctggccttgctgctccacgccgccaggccgcaggtgcagctccagcagtccggcccagagctggagaagcctggcgcctctgtgaagctgagctgtaaggccagcggctactccttcaccggctatacaatgaactgggtgaagcagtcccacggcaagtctctggagtggatcggcctgatcaccccctacaacggcgccagctcctataatcagaagtttcgcggcaaggccaccctgacagtggataagtctagctccaccgcctacatggacctgctgtctctgacaagcgaggattccgccgtgtacttctgcgccagaggcggctatgacggcagaggctttgattactggggccagggcaccacagtgaccgtgtctagcggcgtgggcggctctggaggaggaggcagcggcggaggaggctccgacatcgagctgacacagtccccagcaatcatgtctgccagccccggcgagaaggtgaccatgacatgttccgcctcctctagcgtgtcttacatgcactggtatcagcagaagtctggcaccagccctaagaggtggatctatgatacaagcaagctggcatccggcgtgccaggccgcttctccggctctggcagcggcaattcctactctctgaccatctcctctgtggaggccgaggacgatgccacatactattgccagcagtggagcaagcacccactgacctttggcgccggcacaaagctggagatcaagactagtggcggcggaggctctggcggcggcggcagcggcggcggaggctccgctagcgtggagaaggagcaccctcagctgggagcaggcaccgtgctgctgctgagggccggcttctatgccgtgagctttctgtccgtggccgtgggctccaccgtgtactatcagggcaagtgcctgacatggaaaggcccccggagacagctgccagccgtggtgccagcaccactgcctccaccctgtggctcctctgcccacctgctgcctccagtgcccggcggctacttcctgggccggctggtccctcgggggcgaggggctgcggaggcagcgacccggaaacagcgtatcactgagaccgagtcgccttatcaggagctccagggtcagaggtcggatgtctacagcgacctcaacacacagaggccgtattacaaa

SEQ ID NO: 88 - DNA, 207 bp, synthetic construct; identical to SEQ ID NO: 67
  source 1..207: mol_type = other DNA
  misc_feature 1..207: note = transmembrane domain of CD8 (DNA sequence)

SEQ ID NO: 89 - DNA, 336 bp, synthetic construct
  source 1..336: mol_type = other DNA
  misc_feature 1..336: note = CD3zeta signaling domain (DNA sequence)
cgcgtgaaattcagccgcagcgcagatgctccagcctacaagcaggggcagaaccagctctacaacgaactcaatcttggtcggagagaggagtacgacgtgctggacaagcggagaggacgggacccagaaatgggcgggaagccgcgcagaaagaatccccaagagggcctgtacaacgagctccaaaaggataagatggcagaagcctatagcgagattggtatgaaaggggaacgcagaagaggcaaaggccacgacggactgtaccagggactcagcaccgccaccaaggacacctatgacgctcttcacatgcaggccctgccgcctcgg

SEQ ID NO: 90 - DNA, 1479 bp, synthetic construct
  source 1..1479: mol_type = other DNA
  misc_feature 1..1479: note = the nucleic acid molecule of comparative example 2
atcgatgccaccatcgatgccaccatggccttaccagtgaccgccttgctcctgccgctggccttgctgctccacgccgccaggccgcaggtgcagctccagcagtccggcccagagctggagaagcctggcgcctctgtgaagctgagctgtaaggccagcggctactccttcaccggctatacaatgaactgggtgaagcagtcccacggcaagtctctggagtggatcggcctgatcaccccctacaacggcgccagctcctataatcagaagtttcgcggcaaggccaccctgacagtggataagtctagctccaccgcctacatggacctgctgtctctgacaagcgaggattccgccgtgtacttctgcgccagaggcggctatgacggcagaggctttgattactggggccagggcaccacagtgaccgtgtctagcggcgtgggcggctctggaggaggaggcagcggcggaggaggctccgacatcgagctgacacagtccccagcaatcatgtctgccagccccggcgagaaggtgaccatgacatgttccgcctcctctagcgtgtcttacatgcactggtatcagcagaagtctggcaccagccctaagaggtggatctatgatacaagcaagctggcatccggcgtgccaggccgcttctccggctctggcagcggcaattcctactctctgaccatctcctctgtggaggccgaggacgatgccacatactattgccagcagtggagcaagcacccactgacctttggcgccggcacaaagctggagatcaagaccactaccccagcaccgaggccacccaccccggctcctaccatcgcctcccagcctctgtccctgcgtccggaggcatgtagacccgcagctggtggggccgtgcatacccggggtcttgacttcgcctgcgatatctacatttgggcccctctggctggtacttgcggggtcctgctgctttcactcgtgatcactctttactgtaagcgcggtcggaagaagctgctgtacatctttaagcaacccttcatgaggcctgtgcagactactcaagaggaggacggctgttcatgccggttcccagaggaggaggaaggcggctgcgaactgcgcgtgaaattcagccgcagcgcagatgctccagcctacaagcaggggcagaaccagctctacaacgaactcaatcttggtcggagagaggagtacgacgtgctggacaagcggagaggacgggacccagaaatgggcgggaagccgcgcagaaagaatccccaagagggcctgtacaacgagctccaaaaggataagatggcagaagcctatagcgagattggtatgaaaggggaacgcagaagaggcaaaggccacgacggactgtaccagggactcagcaccgccaccaaggacacctatgacgctcttcacatgcaggccctgccgcctcggtaa

SEQ ID NO: 91 - DNA, 738 bp, synthetic construct
  source 1..738: mol_type = other DNA
  misc_feature 1..738: note = m971 sfcv
caggtacagctgcagcagtcaggtccaggactggtgaagccctcgcagaccctctcactcacctgtgccatctccggggacagtgtctctagcaacagtgctgcttggaactggatcaggcagtccccatcgagaggccttgagtggctgggaaggacatactacaggtccaagtggtataatgattatgcagtatctgtgaaaagtcgaataaccatcaacccagacacatccaagaaccagttctccctgcagctgaactctgtgactcccgaggacacggctgtgtattactgtgcaagagaagtgactggggatctcgaggatgcttttgatatctggggccaagggacaatggtcaccgtctcctctggaggaggaggatccggaggaggaggaagcggaggaggaggaagcgacatccagatgacccagtctccatcgtccctgtctgcatctgtaggagacagagtcaccatcacttgccgggcaagccagaccatttggagctacttaaattggtatcagcagagaccagggaaagcccctaacctcctgatctatgctgcatccagtttgcaaagtggggtcccatcaaggttcagtggcaggggatctgggacagatttcactctcaccatcagcagtctgcaagctgaagattttgcaacttactactgtcaacagagttacagtatccctcagacttttggccaggggaccaagctggagatcaaa

SEQ ID NO: 92 - DNA, 1746 bp, synthetic construct
  source 1..1746: mol_type = other DNA
  misc_feature 1..1746: note = the nucleic acid molecule of example 3
atgattccagcagtggtcttgctcttactccttttggttgaacaagcagcggccctgggagagcctcagctctgctatatcctggatgccatcctgtttctgtatggaattgtcctcaccctcctctactgtcgactgaagatccaagtgcgaaaggcagctataaccagctatgagaaatcagatggtgtttacacgggcctgagcaccaggaaccaggagacttacgagactctgaagcatgagaaaccaccacagatgattccagcagtggtcttgctcttactccttttggttgaacaagcagcggccctgggagagcctcagctctgctatatcctggatgccatcctgtttctgtatggaattgtcctcaccctcctctactgtcgactgaagatccaagtgcgaaaggcagctataaccagctatgagaaatcagatggtgtttacacgggcctgagcaccaggaaccaggagacttacgagactctgaagcatgagaaaccaccacagggctctggagagggaagaggcagcctgctgacctgcggcgacgtggaggagaatcctggcccaatcgatgccaccatcgatgccaccatggccttaccagtgaccgccttgctcctgccgctggccttgctgctccacgccgccaggccgcaggtacagctgcagcagtcaggtccaggactggtgaagccctcgcagaccctctcactcacctgtgccatctccggggacagtgtctctagcaacagtgctgcttggaactggatcaggcagtccccatcgagaggccttgagtggctgggaaggacatactacaggtccaagtggtataatgattatgcagtatctgtgaaaagtcgaataaccatcaacccagacacatccaagaaccagttctccctgcagctgaactctgtgactcccgaggacacggctgtgtattactgtgcaagagaagtgactggggatctcgaggatgcttttgatatctggggccaagggacaatggtcaccgtctcctctggaggaggaggatccggaggaggaggaagcggaggaggaggaagcgacatccagatgacccagtctccatcgtccctgtctgcatctgtaggagacagagtcaccatcacttgccgggcaagccagaccatttggagctacttaaattggtatcagcagagaccagggaaagcccctaacctcctgatctatgctgcatccagtttgcaaagtggggtcccatcaaggttcagtggcaggggatctgggacagatttcactctcaccatcagcagtctgcaagctgaagattttgcaacttactactgtcaacagagttacagtatccctcagacttttggccaggggaccaagctggagatcaaaattgaagttatgtatcctcctccttacctagacaatgagaagagcaatggaaccattatccatgtgaaagggaaacacctttgtccaagtcccctatttcccggaccttctaagcccgtggagaaggagcaccctcagctgggagcaggcaccgtgctgctgctgagggccggcttctatgccgtgagctttctgtccgtggccgtgggctccaccgtgtactatcagggcaagtgcctgacatggaaaggcccccggagacagctgccagccgtggtgccagcaccactgcctccaccctgtggctcctctgcccacctgctgcctccagtgcccggcggc

SEQ ID NO: 93 - DNA, 1497 bp, synthetic construct
  source 1..1497: mol_type = other DNA
  misc_feature 1..1497: note = the nucleic acid molecule of comparative example 3-1
atcgatgccaccatcgatgccaccatggccttaccagtgaccgccttgctcctgccgctggccttgctgctccacgccgccaggccgcaggtacagctgcagcagtcaggtccaggactggtgaagccctcgcagaccctctcactcacctgtgccatctccggggacagtgtctctagcaacagtgctgcttggaactggatcaggcagtccccatcgagaggccttgagtggctgggaaggacatactacaggtccaagtggtataatgattatgcagtatctgtgaaaagtcgaataaccatcaacccagacacatccaagaaccagttctccctgcagctgaactctgtgactcccgaggacacggctgtgtattactgtgcaagagaagtgactggggatctcgaggatgcttttgatatctggggccaagggacaatggtcaccgtctcctctggaggaggaggatccggaggaggaggaagcggaggaggaggaagcgacatccagatgacccagtctccatcgtccctgtctgcatctgtaggagacagagtcaccatcacttgccgggcaagccagaccatttggagctacttaaattggtatcagcagagaccagggaaagcccctaacctcctgatctatgctgcatccagtttgcaaagtggggtcccatcaaggttcagtggcaggggatctgggacagatttcactctcaccatcagcagtctgcaagctgaagattttgcaacttactactgtcaacagagttacagtatccctcagacttttggccaggggaccaagctggagatcaaaaccactaccccagcaccgaggccacccaccccggctcctaccatcgcctcccagcctctgtccctgcgtccggaggcatgtagacccgcagctggtggggccgtgcatacccggggtcttgacttcgcctgcgatatctacatttgggcccctctggctggtacttgcggggtcctgctgctttcactcgtgatcactctttactgtaagcgcggtcggaagaagctgctgtacatctttaagcaacccttcatgaggcctgtgcagactactcaagaggaggacggctgttcatgccggttcccagaggaggaggaaggcggctgcgaactgcgcgtgaaattcagccgcagcgcagatgctccagcctacaagcaggggcagaaccagctctacaacgaactcaatcttggtcggagagaggagtacgacgtgctggacaagcggagaggacgggacccagaaatgggcgggaagccgcgcagaaagaatccccaagagggcctgtacaacgagctccaaaaggataagatggcagaagcctatagcgagattggtatgaaaggggaacgcagaagaggcaaaggccacgacggactgtaccagggactcagcaccgccaccaaggacacctatgacgctcttcacatgcaggccctgccgcctcggtaa

SEQ ID NO: 94 - DNA, 1488 bp, synthetic construct
  source 1..1488: mol_type = other DNA
  misc_feature 1..1488: note = the nucleic acid molecule of comparative example 3-2
atgattccagcagtggtcttgctcttactccttttggttgaacaagcagcggccctgggagagcctcagctctgctatatcctggatgccatcctgtttctgtatggaattgtcctcaccctcctctactgtcgactgaagatccaagtgcgaaaggcagctataaccagctatgagaaatcagatggtgtttacacgggcctgagcaccaggaaccaggagacttacgagactctgaagcatgagaaaccaccacagggctctggagagggaagaggcagcctgctgacctgcggcgacgtggaggagaatcctggcccaatcgatgccaccatcgatgccaccatggccttaccagtgaccgccttgctcctgccgctggccttgctgctccacgccgccaggccgcaggtacagctgcagcagtcaggtccaggactggtgaagccctcgcagaccctctcactcacctgtgccatctccggggacagtgtctctagcaacagtgctgcttggaactggatcaggcagtccccatcgagaggccttgagtggctgggaaggacatactacaggtccaagtggtataatgattatgcagtatctgtgaaaagtcgaataaccatcaacccagacacatccaagaaccagttctccctgcagctgaactctgtgactcccgaggacacggctgtgtattactgtgcaagagaagtgactggggatctcgaggatgcttttgatatctggggccaagggacaatggtcaccgtctcctctggaggaggaggatccggaggaggaggaagcggaggaggaggaagcgacatccagatgacccagtctccatcgtccctgtctgcatctgtaggagacagagtcaccatcacttgccgggcaagccagaccatttggagctacttaaattggtatcagcagagaccagggaaagcccctaacctcctgatctatgctgcatccagtttgcaaagtggggtcccatcaaggttcagtggcaggggatctgggacagatttcactctcaccatcagcagtctgcaagctgaagattttgcaacttactactgtcaacagagttacagtatccctcagacttttggccaggggaccaagctggagatcaaaattgaagttatgtatcctcctccttacctagacaatgagaagagcaatggaaccattatccatgtgaaagggaaacacctttgtccaagtcccctatttcccggaccttctaagcccgtggagaaggagcaccctcagctgggagcaggcaccgtgctgctgctgagggccggcttctatgccgtgagctttctgtccgtggccgtgggctccaccgtgtactatcagggcaagtgcctgacatggaaaggcccccggagacagctgccagccgtggtgccagcaccactgcctccaccctgtggctcctctgcccacctgctgcctccagtgcccggcggc

SEQ ID NO: 95 - DNA, 2208 bp, Homo sapiens
  source 1..2208: mol_type = genomic DNA
  misc_feature 1..2208: note = truncated CD22 fragment (DNA sequence)
atgcatctcctcggcccctggctcctgctcctggttctagaatacttggctttctctgactcaagtaaatgggtttttgagcaccctgaaaccctctacgcctgggagggggcctgcgtctggatcccctgcacctacagagccctagatggtgacctggaaagcttcatcctgttccacaatcctgagtataacaagaacacctcgaagtttgatgggacaagactctatgaaagcacaaaggatgggaaggttccttctgagcagaaaagggtgcaattcctgggagacaagaataagaactgcacactgagtatccacccggtgcacctcaatgacagtggtcagctggggctgaggatggagtccaagactgagaaatggatggaacgaatacacctcaatgtctctgaaaggccttttccacctcatatccagctccctccagaaattcaagagtcccaggaagtcactctgacctgcttgctgaatttctcctgctatgggtatccgatccaattgcagtggctcctagagggggttccaatgaggcaggctgctgtcacctcgacctccttgaccatcaagtctgtcttcacccggagcgagctcaagttctccccacagtggagtcaccatgggaagattgtgacctgccagcttcaggatgcagatgggaagttcctctccaatgacacggtgcagctgaacgtgaagcacaccccgaagttggagatcaaggtcactcccagtgatgccatagtgagggagggggactctgtgaccatgacctgcgaggtcagcagcagcaacccggagtacacgacggtatcctggctcaaggatgggacctcgctgaagaagcagaatacattcacgctaaacctgcgcgaagtgaccaaggaccagagtgggaagtactgctgtcaggtctccaatgacgtgggcccgggaaggtcggaagaagtgttcctgcaagtgcagtatgccccggaaccttccacggttcagatcctccactcaccggctgtggagggaagtcaagtcgagtttctttgcatgtcactggccaatcctcttccaacaaattacacgtggtaccacaatgggaaagaaatgcagggaaggacagaggagaaagtccacatcccaaagatcctcccctggcacgctgggacttattcctgtgtggcagaaaacattcttggtactggacagaggggcccgggagctgagctggatgtccagtatcctcccaagaaggtgaccacagtgattcaaaaccccatgccgattcgagaaggagacacagtgaccctttcctgtaactacaattccagtaaccccagtgttacccggtatgaatggaaaccccatggcgcctgggaggagccatcgcttggggtgctgaagatccaaaacgttggctgggacaacacaaccatcgcctgcgcagcttgtaatagttggtgctcgtgggcctcccctgtcgccctgaatgtccagtatgccccccgagacgtgagggtccggaaaatcaagcccctttccgagattcactctggaaactcggtcagcctccaatgtgacttctcaagcagccaccccaaagaagtccagttcttctgggagaaaaatggcaggcttctggggaaagaaagccagctgaattttgactccatctccccagaagatgctgggagttacagctgctgggtgaacaactccataggacagacagcgtccaaggcctggacacttgaagtgctgtatgcacccaggaggctgcgtgtgtccatgagcccgggggaccaagtgatggaggggaagagtgcaaccctgacctgtgagagcgacgccaaccctcccgtctcccactacacctggtttgactggaataaccaaagcctcccctaccacagccagaagctgagattggagccggtgaaggtccagcactcgggtgcctactggtgccaggggaccaacagtgtgggcaagggccgttcgcctctcagcaccctcaccgtctactatagcccggagaccatcggcaggcgagtggctgtgggactcgggtcctgcctcgccatcctcatcctggcaatctgtgggctcaagctccagcgacgttggaagaggacacagagccagcaggggcttcaggagaattccagcggccagagcttctttgtgaggaataaaaag

SEQ ID NO: 96 - DNA, 726 bp, synthetic construct
  source 1..726: mol_type = other DNA
  misc_feature 1..726: note = FMC63 scfv (DNA sequence)
gacatccagatgacacagactacatcctccctgtctgcctctctgggagacagagtcaccatcagttgcagggcaagtcaggacattagtaaatatttaaattggtatcagcagaaaccagatggaactgttaaactcctgatctaccatacatcaagattacactcaggagtcccatcaaggttcagtggcagtgggtctggaacagattattctctcaccattagcaacctggagcaagaagatattgccacttacttttgccaacagggtaatacgcttccgtacacgttcggaggggggaccaagctggagatcacaggtggcggtggctcgggcggtggtgggtcgggtggcggcggatctgaggtgaaactgcaggagtcaggacctggcctggtggcgccctcacagagcctgtccgtcacatgcactgtctcaggggtctcattacccgactatggtgtaagctggattcgccagcctccacgaaagggtctggagtggctgggagtaatatggggtagtgaaaccacatactataattcagctctcaaatccagactgaccatcatcaaggacaactccaagagccaagttttcttaaaaatgaacagtctgcaaactgatgacacagccatttactactgtgccaaacattattactacggtggtagctatgctatggactactggggccaaggaacctcagtcaccgtctcctca

SEQ ID NO: 97 - DNA, 1551 bp, synthetic construct
  source 1..1551: mol_type = other DNA
  misc_feature 1..1551: note = the nucleic acid molecule of example 4
atgattccagcagtggtcttgctcttactccttttggttgaacaagcagcggccctgggagagcctcagctctgctatatcctggatgccatcctgtttctgtatggaattgtcctcaccctcctctactgtcgactgaagatccaagtgcgaaaggcagctataaccagctatgagaaatcagatggtgtttacacgggcctgagcaccaggaaccaggagacttacgagactctgaagcatgagaaaccaccacagtacttcctgggccggctggtccctcgggggcgaggggctgcggaggcagcgacccggaaacagcgtatcactgagaccgagtcgccttatcaggagctccagggtcagaggtcggatgtctacagcgacctcaacacacagaggccgtattacaaaggctctggagagggaagaggcagcctgctgacctgcggcgacgtggaggagaatcctggcccaatcgatgccaccatcgatgccaccatggccttaccagtgaccgccttgctcctgccgctggccttgctgctccacgccgccaggccggacatccagatgacacagactacatcctccctgtctgcctctctgggagacagagtcaccatcagttgcagggcaagtcaggacattagtaaatatttaaattggtatcagcagaaaccagatggaactgttaaactcctgatctaccatacatcaagattacactcaggagtcccatcaaggttcagtggcagtgggtctggaacagattattctctcaccattagcaacctggagcaagaagatattgccacttacttttgccaacagggtaatacgcttccgtacacgttcggaggggggaccaagctggagatcacaggtggcggtggctcgggcggtggtgggtcgggtggcggcggatctgaggtgaaactgcaggagtcaggacctggcctggtggcgccctcacagagcctgtccgtcacatgcactgtctcaggggtctcattacccgactatggtgtaagctggattcgccagcctccacgaaagggtctggagtggctgggagtaatatggggtagtgaaaccacatactataattcagctctcaaatccagactgaccatcatcaaggacaactccaagagccaagttttcttaaaaatgaacagtctgcaaactgatgacacagccatttactactgtgccaaacattattactacggtggtagctatgctatggactactggggccaaggaacctcagtcaccgtctcctcagagtccaaatatggtcccccatgcccatcatgcccagtggagaaggagcaccctcagctgggagcaggcaccgtgctgctgctgagggccggcttctatgccgtgagctttctgtccgtggccgtgggctccaccgtgtactatcagggcaagtgcctgacatggaaaggcccccggagacagctgccagccgtggtgccagcaccactgcctccaccctgtggctcctctgcccacctgctgcctccagtgcccggcggc

SEQ ID NO: 98 - DNA, 1485 bp, synthetic construct
  source 1..1485: mol_type = other DNA
  misc_feature 1..1485: note = the nucleic acid molecule of comparative example 4
atcgatgccaccatcgatgccaccatggccttaccagtgaccgccttgctcctgccgctggccttgctgctccacgccgccaggccggacatccagatgacacagactacatcctccctgtctgcctctctgggagacagagtcaccatcagttgcagggcaagtcaggacattagtaaatatttaaattggtatcagcagaaaccagatggaactgttaaactcctgatctaccatacatcaagattacactcaggagtcccatcaaggttcagtggcagtgggtctggaacagattattctctcaccattagcaacctggagcaagaagatattgccacttacttttgccaacagggtaatacgcttccgtacacgttcggaggggggaccaagctggagatcacaggtggcggtggctcgggcggtggtgggtcgggtggcggcggatctgaggtgaaactgcaggagtcaggacctggcctggtggcgccctcacagagcctgtccgtcacatgcactgtctcaggggtctcattacccgactatggtgtaagctggattcgccagcctccacgaaagggtctggagtggctgggagtaatatggggtagtgaaaccacatactataattcagctctcaaatccagactgaccatcatcaaggacaactccaagagccaagttttcttaaaaatgaacagtctgcaaactgatgacacagccatttactactgtgccaaacattattactacggtggtagctatgctatggactactggggccaaggaacctcagtcaccgtctcctcaaccactaccccagcaccgaggccacccaccccggctcctaccatcgcctcccagcctctgtccctgcgtccggaggcatgtagacccgcagctggtggggccgtgcatacccggggtcttgacttcgcctgcgatatctacatttgggcccctctggctggtacttgcggggtcctgctgctttcactcgtgatcactctttactgtaagcgcggtcggaagaagctgctgtacatctttaagcaacccttcatgaggcctgtgcagactactcaagaggaggacggctgttcatgccggttcccagaggaggaggaaggcggctgcgaactgcgcgtgaaattcagccgcagcgcagatgctccagcctacaagcaggggcagaaccagctctacaacgaactcaatcttggtcggagagaggagtacgacgtgctggacaagcggagaggacgggacccagaaatgggcgggaagccgcgcagaaagaatccccaagagggcctgtacaacgagctccaaaaggataagatggcagaagcctatagcgagattggtatgaaaggggaacgcagaagaggcaaaggccacgacggactgtaccagggactcagcaccgccaccaaggacacctatgacgctcttcacatgcaggccctgccgcctcggtaa

SEQ ID NO: 99 - DNA, 1026 bp, synthetic construct
  source 1..1026: mol_type = other DNA
  misc_feature 1..1026: note = truncated CD19 fragment (DNA sequence)
atgccacctcctcgcctcctcttcttcctcctcttcctcacccccatggaagtcaggcccgaggaacctctagtggtgaaggtggaagagggagataacgctgtgctgcagtgcctcaaggggacctcagatggccccactcagcagctgacctggtctcgggagtccccgcttaaacccttcttaaaactcagcctggggctgccaggcctgggaatccacatgaggcccctggccatctggcttttcatcttcaacgtctctcaacagatggggggcttctacctgtgccagccggggcccccctctgagaaggcctggcagcctggctggacagtcaatgtggagggcagcggggagctgttccggtggaatgtttcggacctaggtggcctgggctgtggcctgaagaacaggtcctcagagggccccagctccccttccgggaagctcatgagccccaagctgtatgtgtgggccaaagaccgccctgagatctgggagggagagcctccgtgtctcccaccgagggacagcctgaaccagagcctcagccaggacctcaccatggcccctggctccacactctggctgtcctgtggggtaccccctgactctgtgtccaggggccccctctcctggacccatgtgcaccccaaggggcctaagtcattgctgagcctagagctgaaggacgatcgcccggccagagatatgtgggtaatggagacgggtctgttgttgccccgggccacagctcaagacgctggaaagtattattgtcaccgtggcaacctgaccatgtcattccacctggagatcactgctcggccagtactatggcactggctgctgaggactggtggctggaaggtctcagctgtgactttggcttatctgatcttctgcctgtgttcccttgtgggcattcttcatcttcaaagagccctggtcctgaggaggaaaagaaagcgaatgactgaccccaccaggagattcttcaaagtgacgcctcccccaggaagc